European Patent Application EP 4 205 759 A1, published July 5, 2023. Title: Fowl adenovirus subunit vaccine and production method thereof. Applicant: Veterinärmedizinische Universität Wien. The sequence listing filed with the application follows.

SEQUENCE LISTING (25 sequences)

SEQ ID NO: 1 - protein, 441 aa, Artificial Sequence
  peptide
MATSTPHAFSFGQIGSRKRPAGGDGERDASKVPKMQTPAPSATANGNDELDLVYPFWLQNGSTGGGGGGGSGGNPSLNPPFLDPNGPLTVQNNLLKVNTTAPIAVTNKALTLSFDAESLELTNQQQLAVKIDPEGPLKATTEGIQLSVDPTTLEVDDVDWELTVNLDPNGPLDSSATGITVRVDDTLLIDDDGSGQGKELGVHLNPDGPITADQNGLDLEIDNQTLKITPGSAGGVLSVQLKPQGGLNSQSDGIQVVTQNSIEVDNGALDVKVVANGPLSTTPNGLTLNYDTGDFTVNAGTLSILRNPSLVANAYLTSGARTLQQFTAKGENSSQFSFPCAYYLQQWLSDGLIFSSLYLKLDRTRFTGMSSDPSYQNARYFTFWVGGGAAMNLSQLSTPTITPSTTEWTAFAPALNYSGAPAFVYDANPVFTIYFQPNTGR

SEQ ID NO: 2 - protein, 441 aa, Artificial Sequence
  peptide
MATSTPHAFSFGQIGSRKRPAGGDGERDASKVPKMQTPAPSATANGNDELDLVYPFWLQNGSTGGGGGGGSGGNPSLNPPFLDPNGPLTVQNNLLKVNTTAPIAVTNKALTLAYESDSLELTNQQQLAVKIDPEGPLKATTEGIQLSVDPTTLEVDDVDWELTVKLDPDGPLDSSATGITVRVDETLLIEDDGSGQGKELGVNLNPTGPITADDQGLDLEIDNQTLKVNSVTGGGVLAVQLKSQGGLTAQTDGIQVNTQNSITVTNGALDVKVAANGPLESTDTGLTLNYDPGDFTVNAGTLSIIRDPALVANAYLTSGASTLQQFTAKSENSSQFSFPCAYYLQQWLSDGLIFSSLYLKLDRAQFTNMPTGANYQNARYFTFWVGAGTSFNLSTLTEPTITPNTTQWNAFAPALDYSGAPPFIYDASSVVTIYFEPTSGR

SEQ ID NO: 3 - protein, 407 aa, Artificial Sequence
  peptide
MLRAPKRRHSENGQPESEAGPSPAPIKRAKRMVRASQLDLVYPFDYVADPVGGLNPPFLGGSGPLVDQGGQLTLNVTDPIIIKNRSVDLAHDPSLDVNAQGQLAVAVDPEGALDITPDGLDVKVDGVTVMVNDDWELAVKVDPSGGLDSTAGGLGVSVDDTLLVDQGELGVHLNQQGPITADSSGIDLEINPNMFTVNTSTGSGVLELNLKAQGGIQAGSSGVGVSVDESLEIVNNTLEVKPDPSGPLTVSANGLGLKYDSNTLAVTAGALTVVGGGSVSTPIATFVSGSPSLNTYNATIVNSSSHPFSCAYYLQQWNVQGLLFTSLYVKLDSTTMGTRPGDNSSANAKWFTFWVSAYLQQCNPSGIQAGTVSPSTAALADFEPMANRSVSSPWTYSANAYYQPSSG

SEQ ID NO: 4 - protein, 489 aa, Artificial Sequence
  peptide
MAKSTPFTFSMGQHSSRKRPADSENTQNASKVAKTQTSATRAGVDGNDDLNLVYPFWLQNSTSGGGGGGSGGNPSLNPPFIDPNGPLYVQNSLLYVKTTAPIEVENKSLALAYDSSLDVDAQNQLQVKVDAEGPIRISPDGLDIAVDPSTLEVDDEWELTVKLDPAGPISSSSAGINIRVDDTLLIEDDDTAQVKELGVHLNPNGPITADQDGLDLEVDPQTLTVTTSGATGGVLGVLLKPSGGLQTNIQGIGVAVADTLTISSNTVEVKTDPNGSIGSSSNGIAVVTDPAGPLTTSSNGLSLKLTPNGSIQSSSTGLSVQTDPAGPITSGANGLSLSYDTSDFTVSQGMLSIIRNPSTYPDAYLESGTNLLNNYTAYAENSSNYKFNCAYFLQSWYSNGLVTSSLYLKINRDNLNSLPSGQLSENAKYFTFWVPTYESMNLSNVATPTITPSSVPWGAFLPAQNCTSNPAFKYYLTQPPSIYFEPESG

SEQ ID NO: 5 - protein, 83 aa, Artificial Sequence
  peptide
VDTYLPVLTGDWKTSSTYNPGTITLVVRNATIQLQSQSTFTTSVCYNFRCQNSGIFNNNATSGTLTLGPIFYSCPALSTADVS

SEQ ID NO: 6 - protein, 81 aa, Artificial Sequence
  peptide
LESYLPVLTDNWSQTYNPGTVTLCVKTVRVQLRSQGTFSTLVCYNFRCQNTGIFNSNATAGTMTLGPIFFSCPALSTANAP

SEQ ID NO: 7 - protein, 81 aa, Artificial Sequence
  peptide
SVQTFQPVLTGDWDTNTYNPGTVQVCILPQTVVGGQSTFVNMTCYNFRCQNPGIFKVAASSGTFTIGPIFYSCPTNKLTQP

SEQ ID NO: 8 - protein, 72 aa, Artificial Sequence
  peptide
EFQVFTPVVTGAWNPGNIGIRVLPVPVTASGDRYTLLCYSLQCTNSSIFNPANSGTMIVGPVLYSCPAASVP

SEQ ID NO: 9 - protein, 522 aa, Artificial Sequence
  peptide
MATSTPHAFSFGQIGSRKRPAGGDGERDASKVPKMQTPAPSATANGNDELDLVYPFWLQNGSTGGGGGGGSGGNPSLNPPFLDPNGPLTVQNNLLKVNTTAPIAVTNKALTLSFDAESLELTNQQQLAVKIDPEGPLKATTEGIQLSVDPTTLEVDDVDWELTVNLDPNGPLDSSATGITVRVDDTLLIDDDGSGQGKELGVHLNPDGPITADQNGLDLEIDNQTLKITPGSAGGVLSVQLKPQGGLNSQSDGIQVVTQNSIEVDNGALDVKVVANGPLSTTPNGLTLNYDTGDFTVNAGTLSILRNPSLVANAYLTSGARTLQQFTAKGENSSQFSFPCAYYLQQWLSDGLIFSSLYLKLDRTRFTGMSSDPSYQNARYFTFWVGGGAAMNLSQLSTPTITPSTTEWTAFAPALNYSGAPAFVYDANPVFTIYFQPNTGRLESYLPVLTDNWSQTYNPGTVTLCVKTVRVQLRSQGTFSTLVCYNFRCQNTGIFNSNATAGTMTLGPIFFSCPALSTANAP

SEQ ID NO: 10 - protein, 524 aa, Artificial Sequence
  peptide
MATSTPHAFSFGQIGSRKRPAGGDGERDASKVPKMQTPAPSATANGNDELDLVYPFWLQNGSTGGGGGGGSGGNPSLNPPFLDPNGPLTVQNNLLKVNTTAPIAVTNKALTLAYESDSLELTNQQQLAVKIDPEGPLKATTEGIQLSVDPTTLEVDDVDWELTVKLDPDGPLDSSATGITVRVDETLLIEDDGSGQGKELGVNLNPTGPITADDQGLDLEIDNQTLKVNSVTGGGVLAVQLKSQGGLTAQTDGIQVNTQNSITVTNGALDVKVAANGPLESTDTGLTLNYDPGDFTVNAGTLSIIRDPALVANAYLTSGASTLQQFTAKSENSSQFSFPCAYYLQQWLSDGLIFSSLYLKLDRAQFTNMPTGANYQNARYFTFWVGAGTSFNLSTLTEPTITPNTTQWNAFAPALDYSGAPPFIYDASSVVTIYFEPTSGRVDTYLPVLTGDWKTSSTYNPGTITLVVRNATIQLQSQSTFTTSVCYNFRCQNSGIFNNNATSGTLTLGPIFYSCPALSTADVS

SEQ ID NO: 11 - protein, 488 aa, Artificial Sequence
  peptide
MLRAPKRRHSENGQPESEAGPSPAPIKRAKRMVRASQLDLVYPFDYVADPVGGLNPPFLGGSGPLVDQGGQLTLNVTDPIIIKNRSVDLAHDPSLDVNAQGQLAVAVDPEGALDITPDGLDVKVDGVTVMVNDDWELAVKVDPSGGLDSTAGGLGVSVDDTLLVDQGELGVHLNQQGPITADSSGIDLEINPNMFTVNTSTGSGVLELNLKAQGGIQAGSSGVGVSVDESLEIVNNTLEVKPDPSGPLTVSANGLGLKYDSNTLAVTAGALTVVGGGSVSTPIATFVSGSPSLNTYNATIVNSSSHPFSCAYYLQQWNVQGLLFTSLYVKLDSTTMGTRPGDNSSANAKWFTFWVSAYLQQCNPSGIQAGTVSPSTAALADFEPMANRSVSSPWTYSANAYYQPSSGSVQTFQPVLTGDWDTNTYNPGTVQVCILPQTVVGGQSTFVNMTCYNFRCQNPGIFKVAASSGTFTIGPIFYSCPTNKLTQP

SEQ ID NO: 12 - protein, 561 aa, Artificial Sequence
  peptide
MAKSTPFTFSMGQHSSRKRPADSENTQNASKVAKTQTSATRAGVDGNDDLNLVYPFWLQNSTSGGGGGGSGGNPSLNPPFIDPNGPLYVQNSLLYVKTTAPIEVENKSLALAYDSSLDVDAQNQLQVKVDAEGPIRISPDGLDIAVDPSTLEVDDEWELTVKLDPAGPISSSSAGINIRVDDTLLIEDDDTAQVKELGVHLNPNGPITADQDGLDLEVDPQTLTVTTSGATGGVLGVLLKPSGGLQTNIQGIGVAVADTLTISSNTVEVKTDPNGSIGSSSNGIAVVTDPAGPLTTSSNGLSLKLTPNGSIQSSSTGLSVQTDPAGPITSGANGLSLSYDTSDFTVSQGMLSIIRNPSTYPDAYLESGTNLLNNYTAYAENSSNYKFNCAYFLQSWYSNGLVTSSLYLKINRDNLNSLPSGQLSENAKYFTFWVPTYESMNLSNVATPTITPSSVPWGAFLPAQNCTSNPAFKYYLTQPPSIYFEPESGEFQVFTPVVTGAWNPGNIGIRVLPVPVTASGDRYTLLCYSLQCTNSSIFNPANSGTMIVGPVLYSCPAASVP

SEQ ID NO: 13 - DNA, 1323 bp, Artificial Sequence
  nucleotide
atggcgacctcgactcctcacgccttctcctttggccaaatcggctccagaaaacgccctgcgggcggcgatggcgagcgagacgcctccaaagtgccgaaaatgcagacccccgctccgagcgcgaccgccaacggaaatgacgagctggacctggtctaccccttttggctccaaaacggctccaccggaggaggcggcggcggcggttccggtggaaacccgtccctcaacccgccgtttttggaccccaacggacccctgaccgtccaaaacaacctcctgaaggtcaataccacggcccccatcgccgtcaccaataaggccctgacactctcctttgacgcggagagtctcgagctcactaaccaacagcaactggcggtcaaaatcgaccccgaaggacctctgaaagccactaccgagggaatacagctgtcggtcgaccctacgacgttggaggttgatgacgtcgactgggagttaaccgtgaacctcgaccccaacggccccctagattcctcagccacaggaatcacggtcagagtcgatgacaccttgctcatcgatgatgacggttccggtcaaggcaaagaactgggcgtacatcttaaccccgacggacccattacggcagaccaaaacggtctcgacctggaaatcgacaaccagactcttaaaatcacccccggctcggcgggcggtgttctttcggtacagctgaaaccgcagggaggtctgaattcccaatccgatggtatccaggtggtaacccagaacagtatcgaagttgataacggcgcactcgatgttaaggtagtcgctaacggtccactgtctacaactcccaacggtcttaccctaaactacgataccggtgacttcaccgtaaatgccgggaccttaagtatacttcggaacccctctctcgtcgccaatgcctatcttacgtccggggcaagaacactgcaacagttcaccgctaaaggggaaaactctagtcagttttcctttccatgtgcttattatcttcaacagtggttatcggatggactcattttcagttccctctacctaaagttagataggacgcgcttcacagggatgtccagcgatccctcctatcaaaacgccagatatttcacgttctgggtagggggcggcgcggctatgaatctgtcccagttaagtacaccgacgattacccccagtactaccgagtggactgcatttgctcccgccctaaactactccggtgcgcccgccttcgtttatgatgccaatccagtatttacaatctatttccaaccaaacaccgggcga

SEQ ID NO: 14 - DNA, 246 bp, Artificial Sequence
  nucleotide
ctggaaagctatctccccgtccttaccgataactggagccaaacctacaaccccggcaccgtcaccctgtgtgtaaaaacggtaagggttcaattgagatcacaaggaaccttcagcactctagtctgttacaatttccgctgtcagaacacgggcatttttaacagcaacgctacagcgggaaccatgacacttggacctatcttctttagttgtcctgccttaagcaccgccaacgctccttaa

SEQ ID NO: 15 - DNA, 1569 bp, Artificial Sequence
  nucleotide
atggcgacctcgactcctcacgccttctcctttggccaaatcggctccagaaaacgccctgcgggcggcgatggcgagcgagacgcctccaaagtgccgaaaatgcagacccccgctccgagcgcgaccgccaacggaaatgacgagctggacctggtctaccccttttggctccaaaacggctccaccggaggaggcggcggcggcggttccggtggaaacccgtccctcaacccgccgtttttggaccccaacggacccctgaccgtccaaaacaacctcctgaaggtcaataccacggcccccatcgccgtcaccaataaggccctgacactctcctttgacgcggagagtctcgagctcactaaccaacagcaactggcggtcaaaatcgaccccgaaggacctctgaaagccactaccgagggaatacagctgtcggtcgaccctacgacgttggaggttgatgacgtcgactgggagttaaccgtgaacctcgaccccaacggccccctagattcctcagccacaggaatcacggtcagagtcgatgacaccttgctcatcgatgatgacggttccggtcaaggcaaagaactgggcgtacatcttaaccccgacggacccattacggcagaccaaaacggtctcgacctggaaatcgacaaccagactcttaaaatcacccccggctcggcgggcggtgttctttcggtacagctgaaaccgcagggaggtctgaattcccaatccgatggtatccaggtggtaacccagaacagtatcgaagttgataacggcgcactcgatgttaaggtagtcgctaacggtccactgtctacaactcccaacggtcttaccctaaactacgataccggtgacttcaccgtaaatgccgggaccttaagtatacttcggaacccctctctcgtcgccaatgcctatcttacgtccggggcaagaacactgcaacagttcaccgctaaaggggaaaactctagtcagttttcctttccatgtgcttattatcttcaacagtggttatcggatggactcattttcagttccctctacctaaagttagataggacgcgcttcacagggatgtccagcgatccctcctatcaaaacgccagatatttcacgttctgggtagggggcggcgcggctatgaatctgtcccagttaagtacaccgacgattacccccagtactaccgagtggactgcatttgctcccgccctaaactactccggtgcgcccgccttcgtttatgatgccaatccagtatttacaatctatttccaaccaaacaccgggcgactggaaagctatctccccgtccttaccgataactggagccaaacctacaaccccggcaccgtcaccctgtgtgtaaaaacggtaagggttcaattgagatcacaaggaaccttcagcactctagtctgttacaatttccgctgtcagaacacgggcatttttaacagcaacgctacagcgggaaccatgacacttggacctatcttctttagttgtcctgccttaagcaccgccaacgctccttaa

SEQ ID NO: 16 - DNA, 1323 bp, Artificial Sequence
  nucleotide
atggcgacctcgactcctcacgccttctcctttggtcaaatcggctccagaaaacgccctgcgggcggcgatggcgagcgagacgcctccaaagtgccgaaaatgcagacccccgctccgagcgcgaccgccaacggaaatgacgagctggacctggtctaccccttttggctccaaaacggctctaccggaggaggaggcggcggcggttccggtggaaacccgtccctcaacccgccgtttttggaccccaacggacccctgaccgtccaaaacaacctcctgaaggtcaataccacggcgcccatcgccgtcaccaataaggccctgacactcgcctatgaatcggacagtctcgagctcactaaccagcagcaactggcggtcaaaatcgaccccgaaggacctctgaaagccactaccgagggaatacagttgtcggtcgaccctacgacgttggaggttgatgacgtcgactgggagttgacggtgaaactcgaccccgacggccccctggattcctcagccacaggaatcacggtcagagtcgatgagaccttgctcatcgaggatgatgggtccggtcagggcaaagaactcggagtcaatctcaaccccaccggaccgattacggccgatgaccagggtctggacttagaaatagacaaccagacgctcaaggtcaacagtgttaccggcgggggcgtcctagctgtacaactcaaatcccaaggtggtcttaccgcacagactgacggtatccaagtgaacactcagaacagcatcaccgttacaaacggagctctggacgtgaaagtagccgccaacggacctttggagtcaaccgacaccgggctcacactcaactatgaccccggagacttcacagttaatgcgggcacgttgagcattatcagggatccggctctcgtggccaatgcgtacctcacatccggcgcctccacccttcagcaatttacagctaagagtgaaaattccagtcaattttctttcccatgcgcatactatctgcaacagtggctttccgatgggttgatttttagctccctctatctgaagctcgacagagcacagttcacgaacatgccaacgggtgcaaattatcagaacgccaggtactttaccttctgggttggagcgggcacttcatttaatctttctacccttaccgaacccactattacacccaacaccacacaatggaatgcattcgcccctgcccttgattactcaggtgctcctcccttcatctacgacgcgtcttccgtagttacgatttattttgaacccaccagtggtcga

SEQ ID NO: 17 - DNA, 252 bp, Artificial Sequence
  nucleotide
gtggacacatacctgccggttctcaccggcgactggaaaacttcttccacttacaatccaggaacaataacactcgtcgtaaggaacgctacgatccagctgcaatcacagagcacgttcacaaccagtgtgtgttacaacttccgatgtcaaaactctgggattttcaacaacaacgccacctcgggaacgctcaccctaggtccgatcttttacagttgtccggccctaagtactgcggacgtgtcataa

SEQ ID NO: 18 - DNA, 1575 bp, Artificial Sequence
  nucleotide
atggcgacctcgactcctcacgccttctcctttggtcaaatcggctccagaaaacgccctgcgggcggcgatggcgagcgagacgcctccaaagtgccgaaaatgcagacccccgctccgagcgcgaccgccaacggaaatgacgagctggacctggtctaccccttttggctccaaaacggctctaccggaggaggaggcggcggcggttccggtggaaacccgtccctcaacccgccgtttttggaccccaacggacccctgaccgtccaaaacaacctcctgaaggtcaataccacggcgcccatcgccgtcaccaataaggccctgacactcgcctatgaatcggacagtctcgagctcactaaccagcagcaactggcggtcaaaatcgaccccgaaggacctctgaaagccactaccgagggaatacagttgtcggtcgaccctacgacgttggaggttgatgacgtcgactgggagttgacggtgaaactcgaccccgacggccccctggattcctcagccacaggaatcacggtcagagtcgatgagaccttgctcatcgaggatgatgggtccggtcagggcaaagaactcggagtcaatctcaaccccaccggaccgattacggccgatgaccagggtctggacttagaaatagacaaccagacgctcaaggtcaacagtgttaccggcgggggcgtcctagctgtacaactcaaatcccaaggtggtcttaccgcacagactgacggtatccaagtgaacactcagaacagcatcaccgttacaaacggagctctggacgtgaaagtagccgccaacggacctttggagtcaaccgacaccgggctcacactcaactatgaccccggagacttcacagttaatgcgggcacgttgagcattatcagggatccggctctcgtggccaatgcgtacctcacatccggcgcctccacccttcagcaatttacagctaagagtgaaaattccagtcaattttctttcccatgcgcatactatctgcaacagtggctttccgatgggttgatttttagctccctctatctgaagctcgacagagcacagttcacgaacatgccaacgggtgcaaattatcagaacgccaggtactttaccttctgggttggagcgggcacttcatttaatctttctacccttaccgaacccactattacacccaacaccacacaatggaatgcattcgcccctgcccttgattactcaggtgctcctcccttcatctacgacgcgtcttccgtagttacgatttattttgaacccaccagtggtcgagtggacacatacctgccggttctcaccggcgactggaaaacttcttccacttacaatccaggaacaataacactcgtcgtaaggaacgctacgatccagctgcaatcacagagcacgttcacaaccagtgtgtgttacaacttccgatgtcaaaactctgggattttcaacaacaacgccacctcgggaacgctcaccctaggtccgatcttttacagttgtccggccctaagtactgcggacgtgtcataa

SEQ ID NO: 19 - DNA, 35 bp, Artificial Sequence
  nucleotide
aaacctgtattttcagggcatgctccgagccccta

SEQ ID NO: 20 - DNA, 35 bp, Artificial Sequence
  nucleotide
aagtttgcacggatccgctggatggttgatagtat

SEQ ID NO: 21 - DNA, 35 bp, Artificial Sequence
  nucleotide
tccagcgggtccgtgcaaactttccaacccgtatt

SEQ ID NO: 22 - DNA, 35 bp, Artificial Sequence
  nucleotide
gtgagctcgtcgacgtaggttagggttgtgttaat

SEQ ID NO: 23 - DNA, 1221 bp, Artificial Sequence
  nucleotide
atgctccgagcccctaaaagaagacattccgaaaacgggcagcccgagtccgaagcgggaccttccccggctccaatcaagcgcgcgaaacgcatggtgagagcatcccagcttgacctggtttatcctttcgattacgtggccgaccccgtcggagggctcaacccgccttttttgggcggctccggacccctagtggaccagggcggtcagcttacgctcaacgtcaccgatcccatcatcatcaagaacagatcggtggacttggcccacgatcccagtctcgatgtcaacgcccaaggtcaactggcggtggccgttgaccccgaaggggccctggacatcacccccgatggactggacgtcaaggtcgacggagtaaccgtgatggtcaacgatgactgggaactggccgtaaaagtcgacccgtccggcggattggattccactgcgggcggactgggggtcagcgtggacgacaccttgctcgtggatcagggagaactgggcgtacacctcaaccaacaaggacccatcactgccgatagcagtggtatcgacctcgagatcaatcctaacatgttcacggtcaacacctcgaccggaagcggagtgctggaactcaacctaaaagcgcagggaggcatccaagccggcagttcgggagtgggcgtttccgtggatgaaagcctagagattgtcaacaacacgctggaagtgaaaccggatcccagcggaccgcttacggtctccgccaatggcctagggctgaagtacgacagcaataccctggcggtgaccgcgggcgctttgaccgtagtaggagggggaagcgtctccacacccatcgctacttttgtctcgggaagtcccagcctcaacacctacaatgccacgatcgtcaattccagctcgcaccccttctcttgtgcctactaccttcaacagtggaacgtacaagggctcctttttacctccctctacgtgaaactggacagcaccaccatggggactcgccctggggacaacagctccgccaatgccaaatggttcaccttttgggtgtccgcctatctccagcaatgcaacccctccgggattcaagcgggaacggtcagcccctccaccgccgccctcgcggactttgaacccatggccaataggagcgtgtccagcccatggacgtactcggccaatgcatactatcaaccatccagcgga

SEQ ID NO: 24 - DNA, 246 bp, Artificial Sequence
  nucleotide
tccgtgcaaactttccaacccgtattgacaggagattgggataccaacacctacaacccaggaaccgttcaagtctgcatactgcctcaaaccgttgtgggaggccagtcgacctttgttaacatgacatgttataacttccggtgtcaaaatcctggaatattcaaggttgctgctagtagcggcacattcactatcggacccattttctactcctgtccaaccaacaaattaacacaaccctaa

SEQ ID NO: 25 - DNA, 1467 bp, Artificial Sequence
  nucleotide
atgctccgagcccctaaaagaagacattccgaaaacgggcagcccgagtccgaagcgggaccttccccggctccaatcaagcgcgcgaaacgcatggtgagagcatcccagcttgacctggtttatcctttcgattacgtggccgaccccgtcggagggctcaacccgccttttttgggcggctccggacccctagtggaccagggcggtcagcttacgctcaacgtcaccgatcccatcatcatcaagaacagatcggtggacttggcccacgatcccagtctcgatgtcaacgcccaaggtcaactggcggtggccgttgaccccgaaggggccctggacatcacccccgatggactggacgtcaaggtcgacggagtaaccgtgatggtcaacgatgactgggaactggccgtaaaagtcgacccgtccggcggattggattccactgcgggcggactgggggtcagcgtggacgacaccttgctcgtggatcagggagaactgggcgtacacctcaaccaacaaggacccatcactgccgatagcagtggtatcgacctcgagatcaatcctaacatgttcacggtcaacacctcgaccggaagcggagtgctggaactcaacctaaaagcgcagggaggcatccaagccggcagttcgggagtgggcgtttccgtggatgaaagcctagagattgtcaacaacacgctggaagtgaaaccggatcccagcggaccgcttacggtctccgccaatggcctagggctgaagtacgacagcaataccctggcggtgaccgcgggcgctttgaccgtagtaggagggggaagcgtctccacacccatcgctacttttgtctcgggaagtcccagcctcaacacctacaatgccacgatcgtcaattccagctcgcaccccttctcttgtgcctactaccttcaacagtggaacgtacaagggctcctttttacctccctctacgtgaaactggacagcaccaccatggggactcgccctggggacaacagctccgccaatgccaaatggttcaccttttgggtgtccgcctatctccagcaatgcaacccctccgggattcaagcgggaacggtcagcccctccaccgccgccctcgcggactttgaacccatggccaataggagcgtgtccagcccatggacgtactcggccaatgcatactatcaaccatccagcggatccgtgcaaactttccaacccgtattgacaggagattgggataccaacacctacaacccaggaaccgttcaagtctgcatactgcctcaaaccgttgtgggaggccagtcgacctttgttaacatgacatgttataacttccggtgtcaaaatcctggaatattcaaggttgctgctagtagcggcacattcactatcggacccattttctactcctgtccaaccaacaaattaacacaaccctaa